European Patent Application EP 4 438 734 A2, published October 2, 2024. Title: Reprogramming of Cells to a New Fate. Applicant: The Scripps Research Institute. The sequence listing filed with the application follows.

SEQUENCE LISTING (31 sequences)

SEQ ID NO: 1 - protein, 61 aa, synthetic construct
  REGION 1..61: note = synthetic herpes simplex virus structural protein VP22 sequence that enhances transport across membranes
GSPPTAPTRSKTPAQGLARKLHFSTAPPNPDAPWTPRVAGFNKRVFRFSPQTARRATTTRI

SEQ ID NO: 2 - protein, 26 aa, synthetic construct
  REGION 1..26: note = synthetic Kaposi FGF signal sequence (kFGF) that enhances transport across membranes
AGSGGAAVALLPAVLLALLAPGGEFA

SEQ ID NO: 3 - protein, 21 aa, synthetic construct
  REGION 1..21: note = synthetic protein transduction domain-4 (PTD4) sequence that enhances transport across membranes
AGSGGYARAAARQARAGGEFA

SEQ ID NO: 4 - protein, 16 aa, synthetic construct
  REGION 1..16: note = synthetic Penetratin peptide sequence that enhances transport across membranes
RQIKIWFQGRRMKWKK

SEQ ID NO: 5 - protein, 11 aa, synthetic construct
  REGION 1..11: note = synthetic HIV-1 transcriptional activator TAT protein sequence that enhances transport across membranes
YGRKKRRQRRR

SEQ ID NO: 6 - protein, 22 aa, synthetic construct
  REGION 1..22: note = synthetic M918 sequence that enhances transport across membranes
MVTVLFRRLRIRRACGPPRVRV

SEQ ID NO: 7 - protein, 21 aa, synthetic construct
  REGION 1..21: note = synthetic Transportan-10 sequence that enhances transport across membranes
AGYLLGKIGLKALAALAKKIL

SEQ ID NO: 8 - protein, 20 aa, synthetic construct
  REGION 1..20: note = synthetic peptide comprising 11 contiguous arginines that enhances transport across membranes
ESGGGGSPGRRRRRRRRRRR

SEQ ID NO: 9 - protein, 11 aa, synthetic construct
  REGION 1..11: note = synthetic L803 unmyristoylated GSK-3beta Inhibitor XIII
  MOD_RES 10: note = phosphoserine
  MOD_RES 11: note = AMIDATION at C-terminus, prolinamide
KEAPPAPPQSP

SEQ ID NO: 10 - DNA, 24 bp, synthetic construct
  misc_feature 1..24: note = synthetic RT-PCR sense primer for Oct3/4 (Oct4, OCT4) Octamer family transcription factor
  source 1..24: mol_type = other DNA
ggcgttctctttggaaaggtgttc

SEQ ID NO: 11 - DNA, 20 bp, synthetic construct
  misc_feature 1..20: note = synthetic RT-PCR antisense primer for Oct3/4 (Oct4, OCT4) Octamer family transcription factor
  source 1..20: mol_type = other DNA
ctcgaaccacatccttctct

SEQ ID NO: 12 - DNA, 20 bp, synthetic construct
  misc_feature 1..20: note = synthetic RT-PCR sense primer for early-stage cardiac marker Brachyury T (BryT)
  source 1..20: mol_type = other DNA
catgtactctttcttgctgg

SEQ ID NO: 13 - DNA, 20 bp, synthetic construct
  misc_feature 1..20: note = synthetic RT-PCR antisense primer for early-stage cardiac marker Brachyury T (BryT)
  source 1..20: mol_type = other DNA
ggtctcgggaaagcagtggc

SEQ ID NO: 14 - DNA, 24 bp, synthetic construct
  misc_feature 1..24: note = synthetic RT-PCR sense primer for mid-stage cardiac marker GATA4 (GATA-4, Gata-4) zinc-finger transcription factor
  source 1..24: mol_type = other DNA
ttccttgtcctcatcacccacaga

SEQ ID NO: 15 - DNA, 24 bp, synthetic construct
  misc_feature 1..24: note = synthetic RT-PCR antisense primer for mid-stage cardiac marker GATA4 (GATA-4, Gata-4) zinc-finger transcription factor
  source 1..24: mol_type = other DNA
gacaatgttaacgggttgtggagg

SEQ ID NO: 16 - DNA, 24 bp, synthetic construct
  misc_feature 1..24: note = synthetic RT-PCR sense primer for mid-stage cardiac marker Flk1 (Flk-1) receptor for vascular endothelial growth factor (VEGF)
  source 1..24: mol_type = other DNA
ggttctctgtcaagtggcggtaaa

SEQ ID NO: 17 - DNA, 24 bp, synthetic construct
  misc_feature 1..24: note = synthetic RT-PCR antisense primer for mid-stage cardiac marker Flk1 (Flk-1) receptor for vascular endothelial growth factor (VEGF)
  source 1..24: mol_type = other DNA
agcacacaggcagaaaccagtaga

SEQ ID NO: 18 - DNA, 21 bp, synthetic construct
  misc_feature 1..21: note = synthetic RT-PCR sense primer for mid-stage cardiac marker Isl1 (Isl-1, Islet-1)
  source 1..21: mol_type = other DNA
tgtcaggagacttgccacttt

SEQ ID NO: 19 - DNA, 29 bp, synthetic construct
  misc_feature 1..29: note = synthetic RT-PCR antisense primer for mid-stage cardiac marker Isl1 (Isl-1, Islet-1)
  source 1..29: mol_type = other DNA
gccaaacgtttattagtgaaatagtcctg

SEQ ID NO: 20 - DNA, 24 bp, synthetic construct
  misc_feature 1..24: note = synthetic RT-PCR sense primer for mid-stage cardiac marker Nkx2.5 cardiac specific transcription factor
  source 1..24: mol_type = other DNA
acctttctccgatccatcccactt

SEQ ID NO: 21 - DNA, 24 bp, synthetic construct
  misc_feature 1..24: note = synthetic RT-PCR antisense primer for mid-stage cardiac marker Nkx2.5 cardiac specific transcription factor
  source 1..24: mol_type = other DNA
gcgttagcgcactcactttaatgg

SEQ ID NO: 22 - DNA, 24 bp, synthetic construct
  misc_feature 1..24: note = synthetic RT-PCR sense primer for late-stage cardiac marker Mlc2a (Mlc-2a) atrial isoform of myosin light chain
  source 1..24: mol_type = other DNA
aagggaagggtcccatcaacttca

SEQ ID NO: 23 - DNA, 24 bp, synthetic construct
  misc_feature 1..24: note = synthetic RT-PCR antisense primer for late-stage cardiac marker Mlc2a (Mlc-2a) atrial isoform of myosin light chain
  source 1..24: mol_type = other DNA
aacagttgctctacctcagcagga

SEQ ID NO: 24 - DNA, 24 bp, synthetic construct
  misc_feature 1..24: note = synthetic RT-PCR sense primer for Mlc2v (MLC-2v, Myl7) cardiac specific ventricular structural gene
  source 1..24: mol_type = other DNA
acttcaccgtgttcctcacgatgt

SEQ ID NO: 25 - DNA, 24 bp, synthetic construct
  misc_feature 1..24: note = synthetic RT-PCR antisense primer for Mlc2v (MLC-2v, Myl7) cardiac specific ventricular structural gene
  source 1..24: mol_type = other DNA
tccgtgggtaatgatgtggaccaa

SEQ ID NO: 26 - DNA, 20 bp, synthetic construct
  misc_feature 1..20: note = synthetic RT-PCR sense primer for atrial natriuretic factor (ANF)
  source 1..20: mol_type = other DNA
ttcctcgtcttggccttttg

SEQ ID NO: 27 - DNA, 23 bp, synthetic construct
  misc_feature 1..23: note = synthetic RT-PCR antisense primer for atrial natriuretic factor (ANF)
  source 1..23: mol_type = other DNA
cctcatcttctaccggcatcttc

SEQ ID NO: 28 - DNA, 24 bp, synthetic construct
  misc_feature 1..24: note = synthetic RT-PCR sense primer for Nrg1
  source 1..24: mol_type = other DNA
ccaatggccacattgccaataggt

SEQ ID NO: 29 - DNA, 24 bp, synthetic construct
  misc_feature 1..24: note = synthetic RT-PCR antisense primer for Nrg1
  source 1..24: mol_type = other DNA
agcctggcctgtaattcttcctgt

SEQ ID NO: 30 - DNA, 24 bp, synthetic construct
  misc_feature 1..24: note = synthetic RT-PCR sense primer for beta-actin
  source 1..24: mol_type = other DNA
gaaggtgacagcattgcttctgtg

SEQ ID NO: 31 - DNA, 24 bp, synthetic construct
  misc_feature 1..24: note = synthetic RT-PCR antisense primer for beta-actin
  source 1..24: mol_type = other DNA
ttggtctcaagtcagtgtagaggc